European Patent Specification EP 4 087 945 B1, published March 6, 2024. Title: METHODS FOR DETERMINING A LOCATION OF A TARGET NUCLEIC ACID IN A BIOLOGICAL SAMPLE. Applicant: 10x Genomics, Inc Spatial Transcriptomics AB. The sequence listing filed with the application follows.

SEQUENCE LISTING (5 sequences)

SEQ ID NO: 1 - DNA, 10 bp, Artificial
  Poly(dT) Capture Domain
tttttttttt

SEQ ID NO: 2 - DNA, 30 bp, Artificial
  Custom Sequencing Primer
aagcagtggtatcaacgcagagtacatggg

SEQ ID NO: 3 - DNA, 32 bp, Artificial
  Template Switching Oligonucleotide with 10 nt random sequence
  misc_feature (23)..(32): n is a, c, g, or t
aagcagtggtatcaacgcagagnnnnnnnnnn

SEQ ID NO: 4 - DNA, 28 bp, Artificial
  x22_6mer
  misc_feature (23)..(28): n is a, c, g, or t
ttgctaggaccggccttaaagcnnnnnn

SEQ ID NO: 5 - DNA, 32 bp, Artificial
  x22_10mer
  misc_feature (23)..(32): n is a, c, g, or t
ttgctaggaccggccttaaagcnnnnnnnnnn